European Patent Application EP 4 725 500 A2, published April 15, 2026. Title: ANTI-CEACAM5 ANTIBODIES AND CONJUGATES AND USES THEREOF. Applicant: Merck Patent GmbH. Application EP. The sequence listing filed with the application follows.

SEQUENCE LISTING (30 sequences)

SEQ ID NO: 1 - protein, 702 aa, Homo sapiens
  REGION 1..702: note = Human CEACAM5 protein sequence according to GenBank accession number AAA51967.1
MESPSAPPHRWCIPWQRLLLTASLLTFWNPPTTAKLTIESTPFNVAEGKEVLLLVHNLPQHLFGYSWYKGERVDGNRQIIGYVIGTQQATPGPAYSGREIIYPNASLLIQNIIQNDTGFYTLHVIKSDLVNEEATGQFRVYPELPKPSISSNNSKPVEDKDAVAFTCEPETQDATYLWWVNNQSLPVSPRLQLSNGNRTLTLFNVTRNDTASYKCETQNPVSARRSDSVILNVLYGPDAPTISPLNTSYRSGENLNLSCHAASNPPAQYSWFVNGTFQQSTQELFIPNITVNNSGSYTCQAHNSDTGLNRTTVTTITVYAEPPKPFITSNNSNPVEDEDAVALTCEPEIQNTTYLWWVNNQSLPVSPRLQLSNDNRTLTLLSVTRNDVGPYECGIQNELSVDHSDPVILNVLYGPDDPTISPSYTYYRPGVNLSLSCHAASNPPAQYSWLIDGNIQQHTQELFISNITEKNSGLYTCQANNSASGHSRTTVKTITVSAELPKPSISSNNSKPVEDKDAVAFTCEPEAQNTTYLWWVNGQSLPVSPRLQLSNGNRTLTLFNVTRNDARAYVCGIQNSVSANRSDPVTLDVLYGPDTPIISPPDSSYLSGANLNLSCHSASNPSPQYSWRINGIPQQHTQVLFIAKITPNNNGTYACFVSNLATGRNNSIVKSITVSASGTSPGLSAGATVGIMIGVLVGVALI

SEQ ID NO: 2 - protein, 705 aa, Macaca fascicularis
  REGION 1..705: note = Macaca fascicularis CEACAM5 protein sequence (NCBI Reference Sequence XP_005589491.1)
MGSPSAPLHRWCIPWQTLLLTASLLTFWNPPTTAQLTIESRPFNVAEGKEVLLLAHNVSQNLFGYIWYKGERVDASRRIGSCVIRTQQITPGPAHSGRETIDFNASLLIHNVTQSDTGSYTIQVIKEDLVNEEATGQFRVYPELPKPYISSNNSNPVEDKDAVALTCEPETQDTTYLWWVNNQSLPVSPRLELSSDNRTLTVFNIPRNDTTSYKCETQNPVSVRRSDPVTLNVLYGPDAPTISPLNTPYRAGENLNLSCHAASNPTAQYFWFVNGTFQQSTQELFIPNITVNNSGSYMCQAHNSATGLNRTTVTAITVYAELPKPYITSNNSNPIEDKDAVTLTCEPETQDTTYLWWVNNQSLSVSSRLELSNDNRTLTVFNIPRNDTTFYECETQNPVSVRRSDPVTLNVLYGPDAPTISPLNTPYRAGENLNLSCHAASNPAAQYSWFVNGTFQQSTQELFIPNITVNNSGSYMCQAHNSATGLNRTTVTAITVYVELPKPYISSNNSNPIEDKDAVTLTCEPVAENTTYLWWVNNQSLSVSPRLQLSNGNRILTLLSVTRNDTGPYECGIQNSESAKRSDPVTLNVTYGPDTPIISPPDLSYRSGANLNLSCHSDSNPSPQYSWLINGTLRQHTQVLFISKITSNNNGAYACFVSNLATGRNNSIVKNISVSSGDSAPGSSGLSARATVGIIIGMLVGVALM

SEQ ID NO: 3 - protein, 10 aa, synthetic construct
  REGION 1..10: note = CDR1-H of mAb1
DGSVSRGGYY

SEQ ID NO: 4 - protein, 7 aa, synthetic construct
  REGION 1..7: note = CDR2-H of mAb1
IYYSGST

SEQ ID NO: 5 - protein, 11 aa, synthetic construct
  REGION 1..11: note = CDR3-H of mAb1
ARGIAVAPFDY

SEQ ID NO: 6 - protein, 6 aa, synthetic construct
  REGION 1..6: note = CDR1-L of mAb1
QSVRSN

SEQ ID NO: 7 - skipped

SEQ ID NO: 8 - protein, 9 aa, synthetic construct
  REGION 1..9: note = CDR3-L of mAb1
QQYTNWPFT

SEQ ID NO: 9 - protein, 119 aa, synthetic construct
  REGION 1..119: note = VH of mAb1
EVQLQESGPGLVKPSQTLSLTCTVSDGSVSRGGYYLTWIRQHPGKGLEWIGYIYYSGSTYFNPSLRSRVTMSVDTSKNQFSLKLSSVTAADTAVYYCARGIAVAPFDYWGQGTLVTVSS

SEQ ID NO: 10 - protein, 107 aa, synthetic construct
  REGION 1..107: note = VL of mAb1
EIVLTQSPATLSVSPGERATLSCRTSQSVRSNLAWYQQKPGQAPRLLIYAASTRATGIPARFSGSGSGTEFTLTISSLQSEDFAVYYCQQYTNWPFTFGPGTKVDIK

SEQ ID NO: 11 - protein, 328 aa, synthetic construct
  REGION 1..328: note = CH of mAb1
ASTKGPSVFPLAPSSKSTSGGTAALGCLVKDYFPEPVTVSWNSGALTSGVHTFPAVLQSSGLYSLSSVVTVPSSSLGTQTYICNVNHKPSNTKVDKRVEPKSCDKTHTCPPCPAPPVAGPSVFLFPPKPKDTLMISRTPEVTCVVVDVSHEDPEVKFNWYVDGVEVHNAKTKPREEQYNSTYRVVSVLTVLHQDWLNGKEYKCKVSNKALPSSIEKTISKAKGQPREPQVYTLPPSREEMTKNQVSLTCLVKGFYPSDIAVEWESNGQPENNYKTTPPVLDSDGSFFLYSKLTVDKSRWQQGNVFSCSVMHEALHNHYTQKSLSLSPG

SEQ ID NO: 12 - protein, 107 aa, synthetic construct [sequence omitted]

SEQ ID NO: 13 - protein, 447 aa, synthetic construct
  REGION 1..447: note = HC of mAb1
EVQLQESGPGLVKPSQTLSLTCTVSDGSVSRGGYYLTWIRQHPGKGLEWIGYIYYSGSTYFNPSLRSRVTMSVDTSKNQFSLKLSSVTAADTAVYYCARGIAVAPFDYWGQGTLVTVSSASTKGPSVFPLAPSSKSTSGGTAALGCLVKDYFPEPVTVSWNSGALTSGVHTFPAVLQSSGLYSLSSVVTVPSSSLGTQTYICNVNHKPSNTKVDKRVEPKSCDKTHTCPPCPAPPVAGPSVFLFPPKPKDTLMISRTPEVTCVVVDVSHEDPEVKFNWYVDGVEVHNAKTKPREEQYNSTYRVVSVLTVLHQDWLNGKEYKCKVSNKALPSSIEKTISKAKGQPREPQVYTLPPSREEMTKNQVSLTCLVKGFYPSDIAVEWESNGQPENNYKTTPPVLDSDGSFFLYSKLTVDKSRWQQGNVFSCSVMHEALHNHYTQKSLSLSPG

SEQ ID NO: 14 - protein, 214 aa, synthetic construct
  REGION 1..214: note = LC of mAb1
EIVLTQSPATLSVSPGERATLSCRTSQSVRSNLAWYQQKPGQAPRLLIYAASTRATGIPARFSGSGSGTEFTLTISSLQSEDFAVYYCQQYTNWPFTFGPGTKVDIKRTVAAPSVFIFPPSDEQLKSGTASVVCLLNNFYPREAKVQWKVDNALQSGNSQESVTEQDSKDSTYSLSSTLTLSKADYEKHKVYACEVTHQGLSSPVTKSFNRGEC

SEQ ID NO: 15 - DNA, 1404 bp, synthetic construct
  misc_feature 1..1404: note = DNA sequence encoding HC of mAb1
  source 1..1404: mol_type = other DNA
atggagaccgacaccctgctgctgtgggtgctgctgctgtgggtgcccgggtcgaccggtgaggtgcagctgcaggagtcgggcccaggactggtgaagccttcacagaccctgtccctcacctgcactgtctctgatggctccgtcagcaggggtggttactacttgacctggatccgccagcacccagggaagggcctggagtggattgggtacatctattacagtgggagcacctacttcaacccgtccctcaggagtcgggttaccatgtcagtagacacgtctaagaaccagttctccctgaagctgagctctgtgactgccgcggacacggccgtgtattactgtgcgagagggatagcagtggctccctttgactactggggccagggaaccctggtcaccgtctcttcagctagcaccaagggccccagcgtgttccccctggcccccagcagcaagtccacaagcggaggaacagccgccctgggctgcctggtgaaggactacttccccgagcccgtgaccgtgtcctggaacagcggagccctgacctccggcgtgcacaccttccccgccgtgctgcagagcagcggcctgtacagcctgagcagcgtggtgacagtgccaagcagcagcctgggaacccagacctacatctgcaacgtgaaccacaagcccagcaacaccaaggtggacaagagagtggagcccaagagctgcgacaagacccatacctgtccaccctgcccagcccccccagtggccggaccctccgtgttcctgttcccccccaagcccaaggacaccctgatgatcagcaggacccccgaggtgacctgcgtggtggtggacgtgagccacgaggacccagaggtgaagttcaattggtatgtggacggcgtggaggtgcacaacgccaagaccaagcccagagaggaacagtacaacagcacctacagggtggtgtccgtgctgaccgtgctgcaccaggactggctgaacggcaaggaatacaagtgcaaggtctccaacaaggccctgccctccagcatcgagaaaaccatcagcaaggccaagggccagccacgggagccccaggtgtacacactgcccccatctcgggaagaaatgaccaagaaccaggtgtccctgacctgtctggtgaagggcttttaccccagcgacatcgccgtggagtgggagagcaacggccagcccgagaacaactacaagaccaccccccctgtgctggacagcgacggcagcttcttcctgtacagcaagctgaccgtggacaagtccaggtggcagcagggcaacgtgttcagctgcagcgtgatgcacgaggccctgcacaaccactacacacagaagagcctgagcctgtcccccggctga

SEQ ID NO: 16 - DNA, 708 bp, synthetic construct
  misc_feature 1..708: note = DNA sequence encoding LC of mAb1
  source 1..708: mol_type = other DNA
atgagggccctgctggctagactgctgctgtgcgtgctggtcgtgtccgacagcaagggcgaaatcgtactcacgcagtctccagccaccctgtctgtgtctccaggggaaagagccaccctctcctgcaggaccagtcagagtgttcgcagcaacttagcctggtaccagcagaagcctggccaggctcccaggctcctcatctatgctgcatccaccagggccactggtatcccagccaggttcagtggcagtgggtctgggacagagttcactctcaccatcagcagcctgcagtctgaagattttgcagtttattactgtcagcagtatactaactggccattcactttcggccctgggaccaaagtggacatcaaacgtacggtggctgcaccatctgtcttcatcttcccgccatctgatgagcagttgaaatctggaactgcctctgttgtgtgcctgctgaataacttctatcccagagaggccaaagtacagtggaaggtggataacgccctccaatcgggtaactcccaggagagtgtcacagagcaggacagcaaggacagcacctacagcctcagcagcaccctgacgctgagcaaagcagactacgagaaacacaaagtctacgcctgcgaagtcacccatcagggcctgagctcgcccgtcacaaagagcttcaacaggggagagtgttgatag

SEQ ID NO: 17 - protein, 449 aa, synthetic construct
  REGION 1..449: note = HC of antibody hu8G4
EVQLVESGPGLVKPSQTLSLTCTVSDGSVSRGGYYLTWIRQHPGKGLEWIGYIYYSGSTYFNPSLRSRLTMSVDTSKNQFSLKLSSVTAADTAVYYCARGIAVAPFDYWGQGTLVTVSSASTKGPSVFPLAPSSKSTSGGTAALGCLVKDYFPEPVTVSWNSGALTSGVHTFPAVLQSSGLYSLSSVVTVPSSSLGTQTYICNVNHKPSNTKVDKRVEPKSCDKTHTCPPCPAPELLGGPSVFLFPPKPKDTLMISRTPEVTCVVVDVSHEDPEVKFNWYVDGVEVHNAKTKPREEQYNSTYRVVSVLTVLHQDWLNGKEYKCKVSNKALPAPIEKTISKAKGQPREPQVYTLPPSREEMTKNQVSLTCLVKGFYPSDIAVEWESNGQPENNYKTTPPVLDSDGSFFLYSKLTVDKSRWQQGNVFSCSVMHEALHNHYTQKSLSLSPGK

SEQ ID NO: 18 - protein, 214 aa, synthetic construct
  REGION 1..214: note = LC of antibody hu8G4
ETTLTQSPATLSVSPGERATLSCRTSQSVRSNLAWYQQKPGQAPRLLIYAASTRATGIPARFSGSGSGTEFTLTIGSLQSEDFAVYFCQQYTNWPFTFGPGTKVEIKRTVAAPSVFIFPPSDEQLKSGTASVVCLLNNFYPREAKVQWKVDNALQSGNSQESVTEQDSKDSTYSLSSTLTLSKADYEKHKVYACEVTHQGLSSPVTKSFNRGEC

SEQ ID NO: 19 - protein, 449 aa, synthetic construct
  REGION 1..449: note = HC of optimized antibody Variant 1
EVQLQESGPGLVKPSQTLSLTCTVSDGSVSRGGYYLTWIRQHPGKGLEWIGYIYYSGSTYFNPSLRSRLTMSVDTSKNQFSLKLSSVTAADTAVYYCARGIAVAPFDYWGQGTLVTVSSASTKGPSVFPLAPSSKSTSGGTAALGCLVKDYFPEPVTVSWNSGALTSGVHTFPAVLQSSGLYSLSSVVTVPSSSLGTQTYICNVNHKPSNTKVDKRVEPKSCDKTHTCPPCPAPELLGGPSVFLFPPKPKDTLMISRTPEVTCVVVDVSHEDPEVKFNWYVDGVEVHNAKTKPREEQYNSTYRVVSVLTVLHQDWLNGKEYKCKVSNKALPAPIEKTISKAKGQPREPQVYTLPPSREEMTKNQVSLTCLVKGFYPSDIAVEWESNGQPENNYKTTPPVLDSDGSFFLYSKLTVDKSRWQQGNVFSCSVMHEALHNHYTQKSLSLSPGK

SEQ ID NO: 20 - protein, 214 aa, synthetic construct; identical to SEQ ID NO: 18
  REGION 1..214: note = LC of optimized antibody Variant 1

SEQ ID NO: 21 - protein, 214 aa, synthetic construct
  REGION 1..214: note = LC of optimized antibody Variant 2
EIVLTQSPATLSVSPGERATLSCRTSQSVRSNLAWYQQKPGQAPRLLIYAASTRATGIPARFSGSGSGTEFTLTISSLQSEDFAVYFCQQYTNWPFTFGPGTKVDIKRTVAAPSVFIFPPSDEQLKSGTASVVCLLNNFYPREAKVQWKVDNALQSGNSQESVTEQDSKDSTYSLSSTLTLSKADYEKHKVYACEVTHQGLSSPVTKSFNRGEC

SEQ ID NO: 22 - protein, 214 aa, synthetic construct
  REGION 1..214: note = LC of optimized antibody Variant 4
EIVMTQSPATLSVSPGERATLSCRTSQSVRSNLAWYQQKPGQAPRLLIYAASTRATGIPARFSGSGSGTEFTLTISSLQSEDFAVYFCQQYTNWPFTFGPGTKVDIKRTVAAPSVFIFPPSDEQLKSGTASVVCLLNNFYPREAKVQWKVDNALQSGNSQESVTEQDSKDSTYSLSSTLTLSKADYEKHKVYACEVTHQGLSSPVTKSFNRGEC

SEQ ID NO: 23 - protein, 214 aa, synthetic construct
  REGION 1..214: note = LC of optimized antibody Variant 5
EIVMTQSPATLSVSPGERATLSCRTSQSVRSNLAWYQQKPGQAPRLLIYAASTRATGIPARFSGSGSGTEFTLTISSLQSEDFAVYYCQQYTNWPFTFGPGTKVDIKRTVAAPSVFIFPPSDEQLKSGTASVVCLLNNFYPREAKVQWKVDNALQSGNSQESVTEQDSKDSTYSLSSTLTLSKADYEKHKVYACEVTHQGLSSPVTKSFNRGEC

SEQ ID NO: 24 - protein, 449 aa, synthetic construct
  REGION 1..449: note = HC of optimized antibody Variant 6
EVQLQESGPGLVKPSQTLSLTCTVSDGSVSRGGYYLTWIRQHPGKGLEWIGYIYYSGSTYFNPSLRSRVTMSVDTSKNQFSLKLSSVTAADTAVYYCARGIAVAPFDYWGQGTLVTVSSASTKGPSVFPLAPSSKSTSGGTAALGCLVKDYFPEPVTVSWNSGALTSGVHTFPAVLQSSGLYSLSSVVTVPSSSLGTQTYICNVNHKPSNTKVDKRVEPKSCDKTHTCPPCPAPELLGGPSVFLFPPKPKDTLMISRTPEVTCVVVDVSHEDPEVKFNWYVDGVEVHNAKTKPREEQYNSTYRVVSVLTVLHQDWLNGKEYKCKVSNKALPAPIEKTISKAKGQPREPQVYTLPPSREEMTKNQVSLTCLVKGFYPSDIAVEWESNGQPENNYKTTPPVLDSDGSFFLYSKLTVDKSRWQQGNVFSCSVMHEALHNHYTQKSLSLSPGK

SEQ ID NO: 25 - protein, 450 aa, synthetic construct
  REGION 1..450: note = HC of huMab2-3 (allotype)
EVQLQESGPGLVKPGGSLSLSCAASGFVFSSYDMSWVRQTPERGLEWVAYISSGGGITYAPSTVKGRFTVSRDNAKNTLYLQMNSLTSEDTAVYYCAAHYFGSSGPFAYWGQGTLVTVSSASTKGPSVFPLAPSSKSTSGGTAALGCLVKDYFPEPVTVSWNSGALTSGVHTFPAVLQSSGLYSLSSVVTVPSSSLGTQTYICNVNHKPSNTKVDKRVEPKSCDKTHTCPPCPAPELLGGPSVFLFPPKPKDTLMISRTPEVTCVVVDVSHEDPEVKFNWYVDGVEVHNAKTKPREEQYNSTYRVVSVLTVLHQDWLNGKEYKCKVSNKALPAPIEKTISKAKGQPREPQVYTLPPSREEMTKNQVSLTCLVKGFYPSDIAVEWESNGQPENNYKTTPPVLDSDGSFFLYSKLTVDKSRWQQGNVFSCSVMHEALHNHYTQKSLSLSPGK

SEQ ID NO: 26 - protein, 214 aa, synthetic construct
  REGION 1..214: note = LC of huMab2-3
DIQMTQSPASLSASVGDRVTITCRASENIFSYLAWYQQKPGKSPKLLVYNTRTLAEGVPSRFSGSGSGTDFSLTISSLQPEDFATYYCQHHYGTPFTFGSGTKLEIKRTVAAPSVFIFPPSDEQLKSGTASVVCLLNNFYPREAKVQWKVDNALQSGNSQESVTEQDSKDSTYSLSSTLTLSKADYEKHKVYACEVTHQGLSSPVTKSFNRGEC

SEQ ID NO: 27 - protein, 449 aa, synthetic construct
  REGION 1..449: note = HC of hmn-14
EVQLVESGGGVVQPGRSLRLSCSASGFDFTTYWMSWVRQAPGKGLEWIGEIHPDSSTINYAPSLKDRFTISRDNAKNTLFLQMDSLRPEDTGVYFCASLYFGFPWFAYWGQGTPVTVSSASTKGPSVFPLAPSSKSTSGGTAALGCLVKDYFPEPVTVSWNSGALTSGVHTFPAVLQSSGLYSLSSVVTVPSSSLGTQTYICNVNHKPSNTKVDKRVEPKSCDKTHTCPPCPAPELLGGPSVFLFPPKPKDTLMISRTPEVTCVVVDVSHEDPEVKFNWYVDGVEVHNAKTKPREEQYNSTYRVVSVLTVLHQDWLNGKEYKCKVSNKALPAPIEKTISKAKGQPREPQVYTLPPSREEMTKNQVSLTCLVKGFYPSDIAVEWESNGQPENNYKTTPPVLDSDGSFFLYSKLTVDKSRWQQGNVFSCSVMHEALHNHYTQKSLSLSPGK

SEQ ID NO: 28 - protein, 213 aa, synthetic construct
  REGION 1..213: note = LC of hmn-14
DIQLTQSPSSLSASVGDRVTITCKASQDVGTSVAWYQQKPGKAPKLLIYWTSTRHTGVPSRFSGSGSGTDFTFTISSLQPEDIATYYCQQYSLYRSFGQGTKVEIKRTVAAPSVFIFPPSDEQLKSGTASVVCLLNNFYPREAKVQWKVDNALQSGNSQESVTEQDSKDSTYSLSSTLTLSKADYEKHKVYACEVTHQGLSSPVTKSFNRGEC

SEQ ID NO: 29 - protein, 441 aa, synthetic construct
  REGION 1..441: note = HC of rb8G4
EVQLQESGPGLVKPSQTLSLTCTVSDGSVSRGGYYLTWIRQHPGKGLEWIGYIYYSGSTYFNPSLRSRVTMSVDTSKNQFSLKLSSVTAADTAVYYCARGIAVAPFDYWGQGTLVTVSSQPKAPSVFPLAPCCGDTPSSTVTLGCLVKGYLPEPVTVTWNSGTLTNGVRTFPSVRQSSGLYSLSSVVSVTSSSQPVTCNVAHPATNTKVDKTVAPSTCSKPTCPPPELLGGPSVFIFPPKPKDTLMISRTPEVTCVVVDVSEDDPEVQFTWYINNEQVRTARPPLREQQFNSTIRVVSTLPIAHEDWLRGKEFKCKVHNKALPAPIEKTISKARGQPLEPKVYTMGPPREELSSRSVSLTCMINGFYPSDISVEWEKNGKAEDNYKTTPAVLDSDGSYFLYSKLSVPTSEWQRGDVFTCSVMHEALHNHYTQKSISRSPGK

SEQ ID NO: 30 - protein, 213 aa, synthetic construct
  REGION 1..213: note = LC of rb8G4
EIVLTQSPATLSVSPGERATLSCRTSQSVRSNLAWYQQKPGQAPRLLIYAASTRATGIPARFSGSGSGTEFTLTISSLQSEDFAVYYCQQYTNWPFTFGPGTKVDIKRDPVAPSVLLFPPSKEELTTGTATIVCVANKFYPSDITVTWKVDGTTQQSGIENSKTPQSPEDNTYSLSSTLSLTSAQYNSHSVYTCEVVQGSASPIVQSFNRGDC